European Patent Application EP 4 173 485 A1, published May 3, 2023. Title: Protein aggregation inhibiting compounds for plant disease control. Applicant: Max-Planck-Gesellschaft zur Förderung der Wissenschaften e.V. The sequence listing filed with the application follows.

SEQUENCE LISTING (4 sequences)

SEQ ID NO: 1 - DNA, 20 bp, Arabidopsis thaliana
aaggaggctgctgagatgaa

SEQ ID NO: 2 - DNA, 20 bp, Arabidopsis thaliana
tggtggtctcgaacttccag

SEQ ID NO: 3 - DNA, 21 bp, Arabidopsis thaliana
actttcagcagtggatgtcta

SEQ ID NO: 4 - DNA, 21 bp, Arabidopsis thaliana
gatgactcactgaattctgca